European Patent Application EP 4 303 303 A1, published January 10, 2024. Title: ACYCLIC THREONINOL NUCLEIC ACID. Applicant: AGC Inc. The sequence listing filed with the application follows.

SEQUENCE LISTING (2 sequences)

SEQ ID NO: 1 - DNA, 19 bp, Artificial Sequence
  Description of Artificial Sequence: Synthesized control DNA
tttttcagttgaccatata

SEQ ID NO: 2 - DNA, 19 bp, Artificial Sequence
  Description of Artificial Sequence: Synthesized control rDNA
tatatggtcaactgaaaaa